European Patent Application EP 4 534 078 A1, published April 9, 2025. Title: 금나노입자-앱타머 결합체를 기반으로 하는 항균 단백질 전달체 및 이의 제조 방법. Applicant: 엔이에스바이오테크놀러지. The sequence listing filed with the application follows.

SEQUENCE LISTING (4 sequences)

SEQ ID NO: 1 - DNA, 98 bp, synthetic construct
  source 1..98: mol_type = other DNA
aaaacgacggccagtgcgcgcgctttgcttgtgtgagcattgcttttgcattattggtttggttggtgtggttcgtgcgcgccatggtcatagcctgt

SEQ ID NO: 2 - DNA, 80 bp, synthetic construct
  source 1..80: mol_type = other DNA
aaaacgacggccagtctttcgcggggtctggggttggggttgtgggttaattgcacttcgaaatgcatggtcatagctgt

SEQ ID NO: 3 - DNA, 80 bp, synthetic construct
  source 1..80: mol_type = other DNA
aaaacgacggccagtggctggtaggtttgggtggtttggttgggattcggttggttggtaccagccatggtcatagctgt

SEQ ID NO: 4 - DNA, 97 bp, synthetic construct
  source 1..97: mol_type = other DNA
aaaacgacggccagtgcgcgcgctttgcttgtgtgagcattgcttttgcattattggtttggttggtgtggttcgtgcgcgccatggtcatagctgt